European Patent Application EP 4 796 649 A1, published August 26, 2026. Title: IN VITRO METHOD FOR THE DIAGNOSIS AND/OR PROGNOSIS OF PANCREATIC CANCER; AND/OR MONITORING TREATMENT RESPONSE OF PATIENTS SUFFERING FROM PANCREATIC CANCER. Applicant: Servizo Galego de Saúde. The sequence listing filed with the application follows.

SEQUENCE LISTING (18 sequences)

SEQ ID NO: 1 - DNA, 18 bp, synthetic construct
  source 1..18: mol_type = other DNA
gtagtagttgcgttgggc

SEQ ID NO: 2 - DNA, 19 bp, synthetic construct
  source 1..19: mol_type = other DNA
taataaaatcaccgcgttc

SEQ ID NO: 3 - DNA, 24 bp, synthetic construct
  source 1..24: mol_type = other DNA
tataggatcgggtttcgttgggtt

SEQ ID NO: 4 - DNA, 21 bp, synthetic construct
  source 1..21: mol_type = other DNA
taggtagtagttgtgttgggt

SEQ ID NO: 5 - DNA, 22 bp, synthetic construct
  source 1..22: mol_type = other DNA
taataaaatcaccacattccaa

SEQ ID NO: 6 - DNA, 23 bp, synthetic construct
  source 1..23: mol_type = other DNA
tataggattgggttttgttgggt

SEQ ID NO: 7 - DNA, 20 bp, synthetic construct
  source 1..20: mol_type = other DNA
ggtgttaagcgtagttggac

SEQ ID NO: 8 - DNA, 18 bp, synthetic construct
  source 1..18: mol_type = other DNA
ctactacacccgaaaccg

SEQ ID NO: 9 - DNA, 22 bp, synthetic construct
  source 1..22: mol_type = other DNA
ttgggcgagtgatagtttcggt

SEQ ID NO: 10 - DNA, 20 bp, synthetic construct
  source 1..20: mol_type = other DNA
ggtgttaagtgtagttggat

SEQ ID NO: 11 - DNA, 18 bp, synthetic construct
  source 1..18: mol_type = other DNA
ctactacacccaaaacca

SEQ ID NO: 12 - DNA, 23 bp, synthetic construct
  source 1..23: mol_type = other DNA
ttgggtgagtgatagttttggtt

SEQ ID NO: 13 - DNA, 19 bp, synthetic construct
  source 1..19: mol_type = other DNA
gagcgttggtgagtttgtc

SEQ ID NO: 14 - DNA, 20 bp, synthetic construct
  source 1..20: mol_type = other DNA
caacactaaaaaacgaacgc

SEQ ID NO: 15 - DNA, 19 bp, synthetic construct
  source 1..19: mol_type = other DNA
cggagaggacgtagcgttc

SEQ ID NO: 16 - DNA, 21 bp, synthetic construct
  source 1..21: mol_type = other DNA
gtgagtgttggtgagtttgtt

SEQ ID NO: 17 - DNA, 22 bp, synthetic construct
  source 1..22: mol_type = other DNA
acaacactaaaaaacaaacacc

SEQ ID NO: 18 - DNA, 23 bp, synthetic construct
  source 1..23: mol_type = other DNA
tggagaggatgtagtgtttggtt